European Patent Specification EP 3 758 736 B1, published May 1, 2024. Title: USE OF IL-34 TO TREAT RETINAL INFLAMMATION AND NEURODEGENERATION. Applicant: THE UNITED STATES OF AMERICA, as represented by the Secretary, Department of Caspi, Rachel R Mattapallil, Mary  Joseph Wu, Zhijian. The sequence listing filed with the application follows.

SEQUENCE LISTING (9 sequences)

SEQ ID NO: 1 - protein, 242 aa, Homo sapiens
MPRGFTWLRYLGIFLGVALGNEPLEMWPLTQNEECTVTGFLRDKLQYRSRLQYMKHYFPINYKISVPYEGVFRIANVTRLQRAQVSERELRYLWVLVSLSATESVQDVLLEGHPSWKYLQEVETLLLNVQQGLTDVEVSPKVESVLSLLNAPGPNLKLVRPKALLDNCFRVMELLYCSCCKQSSVLNWQDCEVPSPQSCSPEPSLQYAATQLYPPPPWSPSSPPHSTGSVRPVRAQGEGLLP

SEQ ID NO: 2 - protein, 235 aa, Mus musculus
MPWGLAWLYCLGILLDVALGNENLEIWTLTQDKECDLTGYLRGKLQYKNRLQYMKHYFPINYRIAVPYEGVLRVANITRLQKAHVSERELRYLWVLVSLNATESVMDVLLEGHPSWKYLQEVQTLLENVQRSLMDVEIGPHVEAVLSLLSTPGLSLKLVRPKALLDNCFRVMELLYCSCCKQSPILKWQDCELPRLHPHSPGSLMQCTATNVYPLSRQTPTSLPGSPSSSHGSLP

SEQ ID NO: 3 - DNA, 1796 bp, Homo sapiens
catcagacgggaagcctggactgtgggttgggggcagcctcagcctctccaacctggcacccactgcccgtggcccttaggcacctgcttggggtcctggagccccttaaggccaccagcaaatcctaggagaccgagtcttggcacgtgaacagagccagatttcacactgagcagctgcagtcggagaaatcagagaaagcgtcacccagccccagattccgaggggcctgccagggactctctcctcctgctccttggaaaggaagaccccgaaagacccccaagccaccggctcagacctgcttctgggctgccatgggacttgcggccaccgccccccggctgtcctccacgctgccgggcagataagggcagctgctgcccttggggcacctgctcactcccgcagcccagccactcctccagggccagcccttccctgactgagtgaccacctctgctgccccgaggccatgtaggccgtgcttaggcctctgtggacacactgctggggacggcgcctgagctctcagggggacgaggaacaccaccatgccccggggcttcacctggctgcgctatcttgggatcttccttggcgtggccttggggaatgagcctttggagatgtggcccttgacgcagaatgaggagtgcactgtcacgggttttctgcgggacaagctgcagtacaggagccgacttcagtacatgaaacactacttccccatcaactacaagatcagtgtgccttacgagggggtgttcagaatcgccaacgtcaccaggctgcagagggcccaggtgagcgagcgggagctgcggtatctgtgggtcttggtgagcctcagtgccactgagtcggtgcaggacgtgctgctcgagggccacccatcctggaagtacctgcaggaggtggagacgctgctgctgaatgtccagcagggcctcacggatgtggaggtcagccccaaggtggaatccgtgttgtccctcttgaatgccccagggccaaacctgaagctggtgcggcccaaagccctgctggacaactgcttccgggtcatggagctgctgtactgctcctgctgtaaacaaagctccgtcctaaactggcaggactgtgaggtgccaagtcctcagtcttgcagcccagagccctcattgcagtatgcggccacccagctgtaccctccgcccccgtggtcccccagctccccgcctcactccacgggctcggtgaggccggtcagggcacagggcgagggcctcttgccctgagcaccctggatggtgactgcggataggggcagccagaccagctcccacaggagttcaactgggtctgagacttcaaggggtggtggtgggagccccccttgggagaggacccctgggaagggtgtttttcctttgagggggattctgtgccacagcagggctcagcttcctgccttccatagctgtcatggcctcacctggagcggaggggacctggggacctgaaggtggatggggacacagctcctggcttctcctggtgctgccctcactgtccccccgcctaaagggggtactgagcctcctgtggcccgcagcagtgagggcacagctgtgggttgcaggggagacagccagcacggcgtggccattctatgaccccccagcctggcagactggggagctgggggcagagggcggtgccaagtgccacatcttgccatagtggatgctcttccagtttcttttttctattaaacaccccacttcctttggaaaaaaaaaaaaaaaaa

SEQ ID NO: 4 - DNA, 708 bp, Mus musculus
atgccctggggactcgcctggctatactgtcttgggatcctacttgacgtggctttgggaaacgagaatttggagatatggactctgacccaagataaggagtgtgaccttacaggctaccttcggggcaagctgcagtacaagaaccggcttcagtacatgaaacattacttccccatcaactacaggattgctgtgccttatgagggggtactcagagtggccaacatcacaaggctgcagaaggctcacgtgagtgagcgagagcttcggtacctgtgggtcttggtgagtctcaatgccactgagtctgtgatggatgtacttctcgagggccacccgtcctggaagtatctacaggaggttcagacattgctggagaacgtacagcggagcctcatggatgtggagattggccctcacgtggaagctgtgttatctcttctgagtactccaggcctaagcctgaagctggtgcggcccaaagccttgctggacaactgcttccgggtcatggaactgctgtactgttcttgctgtaaacaaagccccatcttaaaatggcaggactgcgagctgcccaggctccatccccacagtccggggtccttgatgcaatgtacagctacaaatgtgtaccctttgtctcggcagacccccacctccctgcccggatccccaagctcaagccatggctcgttgccctga

SEQ ID NO: 5 - protein, 20 aa, Mus musculus
LAQGAYRTAVDLESLASQLT

SEQ ID NO: 6 - DNA, 4771 bp, Artificial Sequence
  pV5.2 CMV mIL-34
ccaactccatcactaggggttcctgcggccgcacgcgtggagctagttattaatagtaatcaattacggggtcattagttcatagcccatatatggagttccgcgttacataacttacggtaaatggcccgcctggctgaccgcccaacgacccccgcccattgacgtcaataatgacgtatgttcccatagtaacgccaatagggactttccattgacgtcaatgggtggagtatttacggtaaactgcccacttggcagtacatcaagtgtatcatatgccaagtacgccccctattgacgtcaatgacggtaaatggcccgcctggcattatgcccagtacatgaccttatgggactttcctacttggcagtacatctagtattagtcatcgctattaccatggtgatgcggttttggcagtacatcaatgggcgtggatagcggtttgactcacggggatttccaagtctccaccccattgacgtcaatgggagtttgttttggcaccaaaatcaacgggactttccaaaatgtcgtaacaactccgccccattgacgcaaatgggcggtaggcgtgtacggtgggaggtctatataagcagagctcgtttagtgaaccgtcagatcgcctggagacgccatccacgctgttttgacctccatagaagacaccgggaccgatccagcctccgcggccgggaacggtgcattggaacgcggattccccgtgccaagagtgacgtaagtaccgcctatagagtctataggcccacccccttgcttttattttttggttgggataaggctggattattctgagtccaagctaggcccttttgctaatcatcttcatacctcttatcttcctcccacagctcctgggcaacgtgctggtctgtgtgctggcccatcactttggcaaagaattatcgatagccaccatgccctggggactcgcctggctatactgtcttgggatcctacttgacgtggctttgggaaacgagaatttggagatatggactctgacccaagataaggagtgtgaccttacaggctaccttcggggcaagctgcagtacaagaaccggcttcagtacatgaaacattacttccccatcaactacaggattgctgtgccttatgagggggtactcagagtggccaacatcacaaggctgcagaaggctcacgtgagtgagcgagagcttcggtacctgtgggtcttggtgagtctcaatgccactgagtctgtgatggatgtacttctcgagggccacccgtcctggaagtatctacaggaggttcagacattgctggagaacgtacagcggagcctcatggatgtggagattggccctcacgtggaagctgtgttatctcttctgagtactccaggcctaagcctgaagctggtgcggcccaaagccttgctggacaactgcttccgggtcatggaactgctgtactgttcttgctgtaaacaaagccccatcttaaaatggcaggactgcgagctgcccaggctccatccccacagtccggggtccttgatgcaatgtacagctacaaatgtgtaccctttgtctcggcagacccccacctccctgcccggatccccaagctcaagccatggctcgttgccctgaagatctaatctcgctttcttgctgtccaatttctattaaaggttcctttgttccctaagtccaactactaaactgggggatattatgaagggccttgagcatctggattctgcctaataaaaaacatttattttcattgcaatgatgtatttaaattatttctgaatattttactaaaaagggaatgtgggaggtcagtgcatttaaaacataaagaaagtaggggcgcgccaggaacccctagtgatggagttggccactccctctctgcgcgctcgctcgctcactgaggccgcccgggcaaagcccgggcgtcgggcgacctttggtcgcccggcctcagtgagcgagcgagcgcgcagagagggagtggccaaggccggccaagcttggcgtaatcatggtcatagctgtttcctgtgtgaaattgttatccgctcacaattccacacaacatacgagccggaagcataaagtgtaaagcctggggtgcctaatgagtgagctaactcacattaattgcgttgcgctcactgcccgctttccagtcgggaaacctgtcgtgccagctgcattaatgaatcggccaagcttcctcgctcactgactcgctgcgctcggtcgttcggctgcggcgagcggtatcagctcactcaaaggcggtaatacggttatccacagaatcaggggataacgcaggaaagaacatgtgagcaaaaggccagcaaaaggccaggaaccgtaaaaaggccgcgttgctggcgtttttccataggctccgcccccctgacgagcatcacaaaaatcgacgctcaagtcagaggtggcgaaacccgacaggactataaagataccaggcgtttccccctggaagctccctcgtgcgctctcctgttccgaccctgccgcttaccggatacctgtccgcctttctcccttcgggaagcgtggcgctttctcatagctcacgctgtaggtatctcagttcggtgtaggtcgttcgctccaagctgggctgtgtgcacgaaccccccgttcagcccgaccgctgcgccttatccggtaactatcgtcttgagtccaacccggtaagacacgacttatcgccactggcagcagccactggtaacaggattagcagagcgaggtatgtaggcggtgctacagagttcttgaagtggtggcctaactacggctacactagaagaacagtatttggtatctgcgctctgctgaagccagttaccttcggaaaaagagttggtagctcttgatccggcaaacaaaccaccgctggtagcggtggtttttttgtttgcaagcagcagattacgcgcagaaaaaaaggatctcaagaagatcctttgatcttttctacggggtctgacgctcagtggaacgaaaactcacgttaagggattttggtcatgagattatcaaaaaggatcttcacctagatccttttaaattaaaaatgaagttttaaatcaatctaaagtatatatgagtaaacttggtctgacagttaccaatgcttaatcagtgaggcacctatctcagcgatctgtctatttcgttcatccatagttgcctgactccccgtcgtgtagataactacgatacgggagggcttaccatctggccccagtgctgcaatgataccgcgagacccacgctcaccggctccagatttatcagcaataaaccagccagccggaagggccgagcgcagaagtggtcctgcaactttatccgcctccatccagtctattaattgttgccgggaagctagagtaagtagttcgccagttaatagtttgcgcaacgttgttgccattgctacaggcatcgtggtgtcacgctcgtcgtttggtatggcttcattcagctccggttcccaacgatcaaggcgagttacatgatcccccatgttgtgcaaaaaagcggttagctccttcggtcctccgatcgttgtcagaagtaagttggccgcagtgttatcactcatggttatggcagcactgcataattctcttactgtcatgccatccgtaagatgcttttctgtgactggtgagtactcaaccaagtcattctgagaatagtgtatgcggcgaccgagttgctcttgcccggcgtcaatacgggataataccgcgccacatagcagaactttaaaagtgctcatcattggaaaacgttcttcggggcgaaaactctcaaggatcttaccgctgttgagatccagttcgatgtaacccactcgtgcacccaactgatcttcagcatcttttactttcaccagcgtttctgggtgagcaaaaacaggaaggcaaaatgccgcaaaaaagggaataagggcgacacggaaatgttgaatactcatactcttcctttttcaatattattgaagcatttatcagggttattgtctcatgagcggatacatatttgaatgtatttagaaaaataaacaaataggggttccgcgcacatttccccgaaaagtgccacctgacgtctaagaaaccattattatcatgacattaacctataaaaataggcgtatcacgaggccctttcgtctcgcgcgtttcggtgatgacggtgaaaacctctgacacatgcagctcccggagacggtcacagcttgtctgtaagcggatgccgggagcagacaagcccgtcagggcgcgtcagcgggtgttggcgggtgtcggggctggcttaactatgcggcatcagagcagattgtactgagagtgcaccatatgcggtgtgaaataccgcacagatgcgtaaggagaaaataccgcatcaggcgccattcgccattcaggctgcgcaactgttgggaagggcgatcggtgcgggcctcttcgctattacgccagctggcgaaagggggatgtgctgcaaggcgattaagttgggtaacgccagggttttcccagtcacgacgttgtaaaacgacggccagtgaattaattcctcgatcgagttaattaacacagctgcgcgctcgctcgctcactgaggccgcccgggcaaagcccgggcgtcgggcgacctttggtcgcccggcctcagtgagcgagcgagcgcgcagagagggagt

SEQ ID NO: 7 - DNA, 334 bp, Artificial Sequence
  Inducible Promoter
atcgatactagactcgagtttactccctatcagtgatagagaacgtatgaagagtttactccctatcagtgatagagaacgtatgcagactttactccctatcagtgatagagaacgtataaggagtttactccctatcagtgatagagaacgtatgaccagtttactccctatcagtgatagagaacgtatctacagtttactccctatcagtgatagagaacgtatatccagtttactccctatcagtgatagagaacgtataagctttaggcgtgtacggtgggcgcctataaaagcagagctcgtttagtgaaccgtcagatcgcctgga

SEQ ID NO: 8 - DNA, 8347 bp, Artificial Sequence
  7m8 vector
gaattcccatcatcaataatataccttattttggattgaagccaatatgataatgagggggtggagtttgtgacgtggcgcggggcgtgggaacggggcgggtgacgtagtagctctagaggtcctgtattagaggtcacgtgagtgttttgcgacattttgcgacaccatgtggtcacgctgggtatttaagcccgagtgagcacgcagggtctccattttgaagcgggaggtttgaacgcgcagccaccacggcggggttttacgagattgtgattaaggtccccagcgaccttgacgagcatctgcccggcatttctgacagctttgtgaactgggtggccgagaaggaatgggagttgccgccagattctgacatggatctgaatctgattgagcaggcacccctgaccgtggccgagaagctgcagcgcgactttctgacggaatggcgccgtgtgagtaaggccccggaggcccttttctttgtgcaatttgagaagggagagagctacttccacatgcacgtgctcgtggaaaccaccggggtgaaatccatggttttgggacgtttcctgagtcagattcgcgaaaaactgattcagagaatttaccgcgggatcgagccgactttgccaaactggttcgcggtcacaaagaccagaaatggcgccggaggcgggaacaaggtggtggatgagtgctacatccccaattacttgctccccaaaacccagcctgagctccagtgggcgtggactaatatggaacagtatttaagcgcctgtttgaatctcacggagcgtaaacggttggtggcgcagcatctgacgcacgtgtcgcagacgcaggagcagaacaaagagaatcagaatcccaattctgatgcgccggtgatcagatcaaaaacttcagccaggtacatggagctggtcgggtggctcgtggacaaggggattacctcggagaagcagtggatccaggaggaccaggcctcatacatctccttcaatgcggcctccaactcgcggtcccaaatcaaggctgccttggacaatgcgggaaagattatgagcctgactaaaaccgcccccgactacctggtgggccagcagcccgtggaggacatttccagcaatcggatttataaaattttggaactaaacgggtacgatccccaatatgcggcttccgtctttctgggatgggccacgaaaaagttcggcaagaggaacaccatctggctgtttgggcctgcaactaccgggaagaccaacatcgcggaggccatagcccacactgtgcccttctacgggtgcgtaaactggaccaatgagaactttcccttcaacgactgtgtcgacaagatggtgatctggtgggaggaggggaagatgaccgccaaggtcgtggagtcggccaaagccattctcggaggaagcaaggtgcgcgtggaccagaaatgcaagtcctcggcccagatagacccgactcccgtgatcgtcacctccaacaccaacatgtgcgccgtgattgacgggaactcaacgaccttcgaacaccagcagccgttgcaagaccggatgttcaaatttgaactcacccgccgtctggatcatgactttgggaaggtcaccaagcaggaagtcaaagactttttccggtgggcaaaggatcacgtggttgaggtggagcatgaattctacgtcaaaaagggtggagccaagaaaagacccgcccccagtgacgcagatataagtgagcccaaacgggtgcgcgagtcagttgcgcagccatcgacgtcagacgcggaagcttcgatcaactacgcagacaggtaccaaaacaaatgttctcgtcacgtgggcatgaatctgatgctgtttccctgcagacaatgcgtgagaatgaatcagaattcaaatatctgcttcactcacggacagaaagactgtttagagtgctttcccgtgtcagaatctcaacccgtttctgtcgtcaaaaaggcgtatcagaaactgtgctacattcatcatatcatgggaaaggtgccagacgcttgcactgcctgcgatctggtcaatgtggatttggatgactgcatctttgaacaataaatgatttaaatcaggtatggctgccgatggttatcttccagattggctcgaggacactctctctgaaggaataagacagtggtggaagctcaaacctggcccaccaccaccaaagcccgcagagcggcataaggacgacagcaggggtcttgtgcttcctgggtacaagtacctcggacccttcaacggactcgacaagggagagccggtcaacgaggcagacgccgcggccctcgagcacgacaaagcctatgaccggcagctcgacagcggagacaacccgtacctcaagtacaaccacgccgacgcggagtttcaggagcgccttaaagaagatacgtcttttgggggcaacctcggacgagcagtcttccaggcgaaaaagagggttcttgaacctctgggcctggttgaggaacctgttaagacggctccgggaaaaaagaggccggtagagcactctcctgtggagccagactcctcctcgggaaccggaaaggcgggccagcagcctgcaagaaaaagattgaattttggtcagactggagacgcagactcagtacctgacccccagcctctcggacagccaccagcagccccctctggtctgggaactaatacgatggctacaggcagtggcgcaccaatggcagacaataacgagggcgccgacggagtgggtaattcctcgggaaattggcattgcgattccacatggatgggcgacagagtcaccaccaccagcacccgaacctgggccctgcccacctacaacaaccacctctacaaacaaatttccagccaatcaggagcctcgaacgacaatcactactttggctacagcaccccttgggggtattttgacttcaacagattccactgccacttttcaccacgtgactggcaaagactcatcaacaacaactggggattccgacccaagagactcaacttcaagctctttaacattcaagtcaaagaggtcacgcagaatgacggtacgacgacgattgccaataaccttaccagcacggttcaggtgtttactgactcggagtaccagctcccgtacgtcctcggctcggcgcatcaaggatgcctcccgccgttcccagcagacgtcttcatggtgccacagtatggatacctcaccctgaacaacgggagtcaggcagtaggacgctcttcattttactgcctggagtactttccttctcagatgctgcgtaccggaaacaactttaccttcagctacacttttgaggacgttcctttccacagcagctacgctcacagccagagtctggaccgtctcatgaatcctctcatcgaccagtacctgtattacttgagcagaacaaacactccaagtggaaccaccacgcagtcaaggcttcagttttctcaggccggagcgagtgacattcgggaccagtctaggaactggcttcctggaccctgttaccgccagcagcgagtatcaaagacatctgcggataacaacaacagtgaatactcgtggactggagctaccaagtaccacctcaatggcagagactctctggtgaatccgggcccggccatggcaagccacaaggacgatgaagaaaagttttttcctcagagcggggttctcatctttgggaagcaaggctcagagaaaacaaatgtggacattgaaaaggtcatgattacagacgaagaggaaatcaggacaaccaatcccgtggctacggagcagtatggttctgtatctaccaacctccagagaggcaacctagcactcggcgaaacaacaagacctgctaggcaagcagctaccgcagatgtcaacacacaaggcgttcttccaggcatggtctggcaggacagagatgtgtaccttcaggggcccatctgggcaaagattccacacacggacggacattttcacccctctcccctcatgggtggattcggacttaaacaccctcctccccagattctcatcaagaacaccccggtacctgcgaatccttcgaccaccttcagtgcggcaaagtttgcttccttcatcacacagtactccacgggacaggtcagcgtggagatcgagtgggagctgcagaaggaaaacagcaaacgctggaatcccgaaattcagtacacttccaactacaacaagtctattaatgtggactttactgtggacactaatggcgtgtattcagagcctcgccccattggcaccagatacctgactcgtaatctgtaattgcggccgcttgttaatcaataaaccgtttaattcgtttcagttgaactttggtctctgcgtatttctttcttatctagtttccatgctctagaggtcctgtattagaggtcacgtgagtgttttgcgacattttgcgacaccatgtggtcacgctgggtatttaagcccgagtgagcacgcagggtctccattttgaagcgggaggtttgaacgcgcagccaccacggcggggttttacgagattgtgattaaggtccccagcgaccttgacgagcatctgcccggcatttctgacagctttgtgaactgggtggccgagaaggaatgggagttgccgccagattctgacatggatctgaatctgattgagcaggcacccctgaccgtggccgagaagctgcatcgctggcgtaatagcgaagaggcccgcaccgatcgcccttcccaacagttgcgcagcctgaatggcgaatggcgattccgttgcaatggctggcggtaatattgttctggatattaccagcaaggccgatagtttgagttcttctactcaggcaagtgatgttattactaatcaaagaagtattgcgacaacggttaatttgcgtgatggacagactcttttactcggtggcctcactgattataaaaacacttctcaggattctggcgtaccgttcctgtctaaaatccctttaatcggcctcctgtttagctcccgctctgattctaacgaggaaagcacgttatacgtgctcgtcaaagcaaccatagtacgcgccctgtagcggcgcattaagcgcggcgggtgtggtggttacgcgcagcgtgaccgctacacttgccagcgccctagcgcccgctcctttcgctttcttcccttcctttctcgccacgttcgccggctttccccgtcaagctctaaatcgggggctccctttagggttccgatttagtgctttacggcacctcgaccccaaaaaacttgattagggtgatggttcacgtagtgggccatcgccctgatagacggtttttcgccctttgacgttggagtccacgttctttaatagtggactcttgttccaaactggaacaacactcaaccctatctcggtctattcttttgatttataagggattttgccgatttcggcatattggttaaaaaatgagctgatttaacaaaaatttaacgcgaattttaacaaaatattaacgcttacaatttaaatatttgcttatacaatcttcctgtttttggggcttttctgattatcaaccggggtacatatgattgacatgctagttttacgattaccgttcatcgattctcttgtttgctccagactctcaggcaatgacctgatagcctttgtagagacctctcaaaaatagctaccctctccggcatgaatttatcagctagaacggttgaatatcatattgatggtgatttgactgtctccggcctttctcacccgtttgaatctttacctacacattactcaggcattgcatttaaaatatatgagggttctaaaaatttttatccttgcgttgaaataaaggcttctcccgcaaaagtattacagggtcataatgtttttggtacaaccgatttagctttatgctctgaggctttattgcttaattttgctaattctttgccttgcctgtatgatttattggatgttggaatcgcctgatgcggtattttctccttacgcatctgtgcggtatttcacaccgcatatggtgcactctcagtacaatctgctctgatgccgcatagttaagccagccccgacacccgccaacacccgctgacgcgccctgacgggcttgtctgctcccggcatccgcttacagacaagctgtgaccgtctccgggagctgcatgtgtcagaggttttcaccgtcatcaccgaaacgcgcgagacgaaagggcctcgtgatacgcctatttttataggttaatgtcatgataataatggtttcttagacgtcaggtggcacttttcggggaaatgtgcgcggaacccctatttgtttatttttctaaatacattcaaatatgtatccgctcatgagacaataaccctgataaatgcttcaataatattgaaaaaggaagagtatgagtattcaacatttccgtgtcgcccttattcccttttttgcggcattttgccttcctgtttttgctcacccagaaacgctggtgaaagtaaaagatgctgaagatcagttgggtgcacgagtgggttacatcgaactggatctcaacagcggtaagatccttgagagttttcgccccgaagaacgttttccaatgatgagcacttttaaagttctgctatgtggcgcggtattatcccgtattgacgccgggcaagagcaactcggtcgccgcatacactattctcagaatgacttggttgagtactcaccagtcacagaaaagcatcttacggatggcatgacagtaagagaattatgcagtgctgccataaccatgagtgataacactgcggccaacttacttctgacaacgatcggaggaccgaaggagctaaccgcttttttgcacaacatgggggatcatgtaactcgccttgatcgttgggaaccggagctgaatgaagccataccaaacgacgagcgtgacaccacgatgcctgtagcaatggcaacaacgttgcgcaaactattaactggcgaactacttactctagcttcccggcaacaattaatagactggatggaggcggataaagttgcaggaccacttctgcgctcggcccttccggctggctggtttattgctgataaatctggagccggtgagcgtgggtctcgcggtatcattgcagcactggggccagatggtaagccctcccgtatcgtagttatctacacgacggggagtcaggcaactatggatgaacgaaatagacagatcgctgagataggtgcctcactgattaagcattggtaactgtcagaccaagtttactcatatatactttagattgatttaaaacttcatttttaatttaaaaggatctaggtgaagatcctttttgataatctcatgaccaaaatcccttaacgtgagttttcgttccactgagcgtcagaccccgtagaaaagatcaaaggatcttcttgagatcctttttttctgcgcgtaatctgctgcttgcaaacaaaaaaaccaccgctaccagcggtggtttgtttgccggatcaagagctaccaactctttttccgaaggtaactggcttcagcagagcgcagataccaaatactgttcttctagtgtagccgtagttaggccaccacttcaagaactctgtagcaccgcctacatacctcgctctgctaatcctgttaccagtggctgctgccagtggcgataagtcgtgtcttaccgggttggactcaagacgatagttaccggataaggcgcagcggtcgggctgaacggggggttcgtgcacacagcccagcttggagcgaacgacctacaccgaactgagatacctacagcgtgagctatgagaaagcgccacgcttcccgaagggagaaaggcggacaggtatccggtaagcggcagggtcggaacaggagagcgcacgagggagcttccagggggaaacgcctggtatctttatagtcctgtcgggtttcgccacctctgacttgagcgtcgatttttgtgatgctcgtcaggggggcggagcctatggaaaaacgccagcaacgcggcctttttacggttcctggccttttgctggccttttgctcacatgttctttcctgcgttatcccctgattctgtggataaccgtattaccgcctttgagtgagctgataccgctcgccgcagccgaacgaccgagcgcagcgagtcagtgagcgaggaagcggaagagcgcccaatacgcaaaccgcctctccccgcg

SEQ ID NO: 9 - DNA, 5244 bp, Artificial Sequence
  pAAV-Tet-On-mIL34 vector
ccaactccatcactaggggttcctgcggccgcacgcgtccatagagcccaccgcatccccagcatgcctgctattgtcttcccaatcctcccccttgctgtcctgccccaccccaccccccagaatagaatgacacctactcagacaatgcgatgcaatttcctcattttattaggaaaggacagtgggagtggcaccttccagggtcaaggaaggcacgggggaggggcaaacaacagatggctggcaactagaaggcacagttacccggggagcatgtcaaggtcaaaatcgtcaagagcgtcagcaggcagcatatcaaggtcaaagtcgtcaagggcatcggctgggagcatgtctaagtcaaaatcgtcaagggcgtcggtcggcccgccgctttcgcactttagctgtttctccaggccacatatgattagttccaggccgaaaaggaaggcaggttcggctccctgccggtcgaacagctcaattgcttgtctcagaagtgggggcatagaatcggtggtaggtgtctctctttcctcttttgctacttgatgctcctgttcctccaatacgcagcccagtgtaaagtggcccacggcggacagagcgtacagtgcgttctccagggagaagccttgctgacacaggaacgcgagctgattttccagggtttcgtactgtttctctgttgggcgggtgccgagatgcactttagccccgtcgcgatgtgagaggagagcacagcggtatgacttggcgttgttccgcagaaagtcttgccatgactcgccttccagggggcagaagtgggtatgatgcctgtccagcatctcgattggcagggcatcgagcagggcccgcttgttcttcacgtgccagtacagggtaggctgctcaactcccagcttttgagcgagtttccttgtcgtcaggccttcgataccgacaccattgagtaattccagagctccgtttatgactttgctcttgtccagtctagacatgcgatctgacggttcactaaacgagctctgcttatataggcctcccaccgtacacgcctacctcgacatacgttctctatcactgatagggagtaaactcgacatacgttctctatcactgatagggataaactcgacatacgttctctatcactgatagggagtaaactcgacatacgttctctatcactgatagggagtaaactcgacatacgttctctatcactgatagggagtaaactcgacatcgttctctatcactgatagggagtaaactcgacatacgttctctatcactgatagggagtaaactcgagtatgtcgaggtggcgtgtacggtgggaggcctatataagcagagctcgtttagtgaaccgtcagatcgccccgcggatcgatagccaccatgccctggggactcgcctggctatactgtcttgggatcctacttgacgtggctttgggaaacgagaatttggagatatggactctgacccaagataaggagtgtgaccttacaggctaccttcggggcaagctgcagtacaagaaccggcttcagtacatgaaacattacttccccatcaactacaggattgctgtgccttatgagggggtactcagagtggccaacatcacaaggctgcagaaggctcacgtgagtgagcgagagcttcggtacctgtgggtcttggtgagtctcaatgccactgagtctgtgatggatgtacttctcgagggccacccgtcctggaagtatctacaggaggttcagacattgctggagaacgtacagcggagcctcatggatgtggagattggccctcacgtggaagctgtgttatctcttctgagtactccaggcctaagcctgaagctggtgcggcccaaagccttgctggacaactgcttccgggtcatggaactgctgtactgttcttgctgtaaacaaagccccatcttaaaatggcaggactgcgagctgcccaggctccatccccacagtccggggtccttgatgcaatgtacagctacaaatgtgtaccctttgtctcggcagacccccacctccctgcccggatccccaagctcaagccatggctcgttgccctgaagatctaatctcgctttcttgctgtccaatttctattaaaggttcctttgttccctaagtccaactactaaactgggggatattatgaagggccttgagcatctggattctgcctaataaaaaacatttattttcattgcaatgatgtatttaaattatttctgaatattttactaaaaagggaatgtgggaggtcagtgcatttaaaacataaagaaagtaggggcgcgccaggaacccctagtgatggagttggccactccctctctgcgcgctcgctcgctcactgaggccgcccgggcaaagcccgggcgtcgggcgacctttggtcgcccggcctcagtgagcgagcgagcgcgcagagagggagtggccaaggccggccaagcttggcgtaatcatggtcatagctgtttcctgtgtgaaattgttatccgctcacaattccacacaacatacgagccggaagcataaagtgtaaagcctggggtgcctaatgagtgagctaactcacattaattgcgttgcgctcactgcccgctttccagtcgggaaacctgtcgtgccagctgcattaatgaatcggccaagcttcctcgctcactgactcgctgcgctcggtcgttcggctgcggcgagcggtatcagctcactcaaaggcggtaatacggttatccacagaatcaggggataacgcaggaaagaacatgtgagcaaaaggccagcaaaaggccaggaaccgtaaaaaggccgcgttgctggcgtttttccataggctccgcccccctgacgagcatcacaaaaatcgacgctcaagtcagaggtggcgaaacccgacaggactataaagataccaggcgtttccccctggaagctccctcgtgcgctctcctgttccgaccctgccgcttaccggatacctgtccgcctttctcccttcgggaagcgtggcgctttctcatagctcacgctgtaggtatctcagttcggtgtaggtcgttcgctccaagctgggctgtgtgcacgaaccccccgttcagcccgaccgctgcgccttatccggtaactatcgtcttgagtccaacccggtaagacacgacttatcgccactggcagcagccactggtaacaggattagcagagcgaggtatgtaggcggtgctacagagttcttgaagtggtggcctaactacggctacactagaagaacagtatttggtatctgcgctctgctgaagccagttaccttcggaaaaagagttggtagctcttgatccggcaaacaaaccaccgctggtagcggtggtttttttgtttgcaagcagcagattacgcgcagaaaaaaaggatctcaagaagatcctttgatcttttctacggggtctgacgctcagtggaacgaaaactcacgttaagggattttggtcatgagattatcaaaaaggatcttcacctagatccttttaaattaaaaatgaagttttaaatcaatctaaagtatatatgagtaaacttggtctgacagttaccaatgcttaatcagtgaggcacctatctcagcgatctgtctatttcgttcatccatagttgcctgactccccgtcgtgtagataactacgatacgggagggcttaccatctggccccagtgctgcaatgataccgcgagacccacgctcaccggctccagatttatcagcaataaaccagccagccggaagggccgagcgcagaagtggtcctgcaactttatccgcctccatccagtctattaattgttgccgggaagctagagtaagtagttcgccagttaatagtttgcgcaacgttgttgccattgctacaggcatcgtggtgtcacgctcgtcgtttggtatggcttcattcagctccggttcccaacgatcaaggcgagttacatgatcccccatgttgtgcaaaaaagcggttagctccttcggtcctccgatcgttgtcagaagtaagttggccgcagtgttatcactcatggttatggcagcactgcataattctcttactgtcatgccatccgtaagatgcttttctgtgactggtgagtactcaaccaagtcattctgagaatagtgtatgcggcgaccgagttgctcttgcccggcgtcaatacgggataataccgcgccacatagcagaactttaaaagtgctcatcattggaaaacgttcttcggggcgaaaactctcaaggatcttaccgctgttgagatccagttcgatgtaacccactcgtgcacccaactgatcttcagcatcttttactttcaccagcgtttctgggtgagcaaaaacaggaaggcaaaatgccgcaaaaaagggaataagggcgacacggaaatgttgaatactcatactcttcctttttcaatattattgaagcatttatcagggttattgtctcatgagcggatacatatttgaatgtatttagaaaaataaacaaataggggttccgcgcacatttccccgaaaagtgccacctgacgtctaagaaaccattattatcatgacattaacctataaaaataggcgtatcacgaggccctttcgtctcgcgcgtttcggtgatgacggtgaaaacctctgacacatgcagctcccggagacggtcacagcttgtctgtaagcggatgccgggagcagacaagcccgtcagggcgcgtcagcgggtgttggcgggtgtcggggctggcttaactatgcggcatcagagcagattgtactgagagtgcaccatatgcggtgtgaaataccgcacagatgcgtaaggagaaaataccgcatcaggcgccattcgccattcaggctgcgcaactgttgggaagggcgatcggtgcgggcctcttcgctattacgccagctggcgaaagggggatgtgctgcaaggcgattaagttgggtaacgccagggttttcccagtcacgacgttgtaaaacgacggccagtgaattaattcctcgatcgagttaattaacacagctgcgcgctcgctcgctcactgaggccgcccgggcaaagcccgggcgtcgggcgacctttggtcgcccggcctcagtgagcgagcgagcgcgcagagagggagtgg